European Patent Application EP 4 410 818 A1, published August 7, 2024. Title: PEPTIDE HAVING ANTI-AGING ACTIVITY, AND USE THEREOF. Applicant: CAREGEN CO., LTD. Application KR. The sequence listing filed with the application follows.

SEQUENCE LISTING (13 sequences)

SEQ ID NO: 1 - protein, 13 aa, synthetic construct
  REGION 1..13: note = peptide
LCACCLHNCNECQ

SEQ ID NO: 2 - DNA, 20 bp, synthetic construct
  misc_feature 1..20: note = Col1a1-F
  source 1..20: mol_type = other DNA
caccctcaagagcctgagtc

SEQ ID NO: 3 - DNA, 20 bp, synthetic construct
  misc_feature 1..20: note = Col1a1-R
  source 1..20: mol_type = other DNA
agacggctgagtagggaaca

SEQ ID NO: 4 - DNA, 20 bp, synthetic construct
  misc_feature 1..20: note = Fibronectin-F
  source 1..20: mol_type = other DNA
ccaggaaccgagtacaccat

SEQ ID NO: 5 - DNA, 20 bp, synthetic construct
  misc_feature 1..20: note = Fibronectin-R
  source 1..20: mol_type = other DNA
atacccaggttgggtgatga

SEQ ID NO: 6 - DNA, 20 bp, synthetic construct
  misc_feature 1..20: note = Elastin-F
  source 1..20: mol_type = other DNA
gcaagacctggctttggact

SEQ ID NO: 7 - DNA, 21 bp, synthetic construct
  misc_feature 1..21: note = Elastin-R
  source 1..21: mol_type = other DNA
gggagtttctggttagggctg

SEQ ID NO: 8 - DNA, 20 bp, synthetic construct
  misc_feature 1..20: note = SIRT1-F
  source 1..20: mol_type = other DNA
tcagtggctggaacagtgag

SEQ ID NO: 9 - DNA, 20 bp, synthetic construct
  misc_feature 1..20: note = SIRT1-R
  source 1..20: mol_type = other DNA
tctggcatgtcccactatca

SEQ ID NO: 10 - DNA, 20 bp, synthetic construct
  misc_feature 1..20: note = AQP3-F
  source 1..20: mol_type = other DNA
ccttcttgggtgctggaata

SEQ ID NO: 11 - DNA, 20 bp, synthetic construct
  misc_feature 1..20: note = AQP3-R
  source 1..20: mol_type = other DNA
acacgataagggaggctgtg

SEQ ID NO: 12 - DNA, 20 bp, synthetic construct
  misc_feature 1..20: note = GAPDH-F
  source 1..20: mol_type = other DNA
ggagccaaaagggtcatcat

SEQ ID NO: 13 - DNA, 20 bp, synthetic construct
  misc_feature 1..20: note = GAPDH-R
  source 1..20: mol_type = other DNA
gtgatggcatggactgtggt